European Patent Application EP 4 729 520 A1, published April 22, 2026. Title: CONFORMATIONALLY FIXED DIPROLINE MIMETICS AND THEIR USE. Applicant: PROSION Therapeutics. Application EP. The sequence listing filed with the application follows.

SEQUENCE LISTING (1 sequence)

SEQ ID NO: 1 - protein, 17 aa, synthetic construct
  VARIANT 8: note = 2-Chlor-L-Phenylalanin
SEPSSFEFPPPPTEDEL